European Patent Application EP 4 349 870 A1, published April 10, 2024. Title: Anti-CD3 Antibody Variant, Fusion Protein, and Application. Applicant: QURE BIOTECHNOLOGY (SHANGHAI) CO., LTD. Application PCT/CN2022/096501. The sequence listing filed with the application follows.

SEQUENCE LISTING (45 sequences)

SEQ ID NO: 1 - protein, 481 aa, Artificial Sequence
  QD3685
EVQLLESGGGLVQPGGSLKLSCAASGFTFNTYAMNWVRQAPGKGLEWVARIRSKYNNYETYYADSVKDRFTISRDDSKNTAYLQMNNLKTEDTAVYYCVRHGNFGNSYVSWFAYWGQGTLVTVSSGGGGSGGGGSGGGGSELVVTQEPSLTVSPGGTVTLTCRSSTGAVTTSNYANWVQQKPGQAPRGLIGGTNLRAPGTPARFSGSLLGGKAALTLSGVQPEDEAEYYCALWRSGGWVFGGGTKLTVLEPKSSDKTHTCPPCPAPELLGGPSVFLFPPKPKDTLMISRTPEVTCVVVDVSHEDPEVKFNWYVDGVEVHNAKTKPREEQYNSTYRVVSVLTVLHQDWLNGKEYKCKVSNKALPAPIEKTISKAKGQPREPQVYTLPPSRDELTKNQVSLTCLVKGFYPSDIAVEWESNGQPENNYKTTPPVLDSDGSFFLYSKLTVDKSRWQQGNVFSCSVMHEALHNHYTQKSLSLSPGK

SEQ ID NO: 2 - protein, 481 aa, Artificial Sequence
  QD3689
EVQLLESGGGLVQPGGSLKLSCAASGFTFNTYAMNWVRQAPGKGLEWVARIRSKYNNYETYYADSVKDRFTISRDDSKNTAYLQMNNLKTEDTAVYYCVRHSNFGNGYVSWFAYWGQGTLVTVSSGGGGSGGGGSGGGGSELVVTQEPSLTVSPGGTVTLTCRSSTGAVTTSNYANWVQQKPGQAPRGLIGGTNLRAPGTPARFSGSLLGGKAALTLSGVQPEDEAEYYCALWNKGGWVFGGGTKLTVLEPKSSDKTHTCPPCPAPELLGGPSVFLFPPKPKDTLMISRTPEVTCVVVDVSHEDPEVKFNWYVDGVEVHNAKTKPREEQYNSTYRVVSVLTVLHQDWLNGKEYKCKVSNKALPAPIEKTISKAKGQPREPQVYTLPPSRDELTKNQVSLTCLVKGFYPSDIAVEWESNGQPENNYKTTPPVLDSDGSFFLYSKLTVDKSRWQQGNVFSCSVMHEALHNHYTQKSLSLSPGK

SEQ ID NO: 3 - protein, 481 aa, Artificial Sequence
  QD3690
EVQLLESGGGLVQPGGSLKLSCAASGFTFNTYAMNWVRQAPGKGLEWVARIRSKYNNYETYYADSVKDRFTISRDDSKNTAYLQMNNLKTEDTAVYYCVRHSNFGNGYVSWFAYWGQGTLVTVSSGGGGSGGGGSGGGGSELVVTQEPSLTVSPGGTVTLTCRSSTGAVTTSNYANWVQQKPGQAPRGLIGGTWLRAPGTPARFSGSLLGGKAALTLSGVQPEDEAEYYCALWNSGGWVFGGGTKLTVLEPKSSDKTHTCPPCPAPELLGGPSVFLFPPKPKDTLMISRTPEVTCVVVDVSHEDPEVKFNWYVDGVEVHNAKTKPREEQYNSTYRVVSVLTVLHQDWLNGKEYKCKVSNKALPAPIEKTISKAKGQPREPQVYTLPPSRDELTKNQVSLTCLVKGFYPSDIAVEWESNGQPENNYKTTPPVLDSDGSFFLYSKLTVDKSRWQQGNVFSCSVMHEALHNHYTQKSLSLSPGK

SEQ ID NO: 4 - protein, 481 aa, Artificial Sequence
  QD3679 (hSP34 VH-VL-FC)
EVQLLESGGGLVQPGGSLKLSCAASGFTFNTYAMNWVRQAPGKGLEWVARIRSKYNNYATYYADSVKDRFTISRDDSKNTAYLQMNNLKTEDTAVYYCVRHGNFGNSYVSWFAYWGQGTLVTVSSGGGGSGGGGSGGGGSELVVTQEPSLTVSPGGTVTLTCRSSTGAVTTSNYANWVQQKPGQAPRGLIGGTNKRAPGTPARFSGSLLGGKAALTLSGVQPEDEAEYYCALWYSNLWVFGGGTKLTVLEPKSSDKTHTCPPCPAPELLGGPSVFLFPPKPKDTLMISRTPEVTCVVVDVSHEDPEVKFNWYVDGVEVHNAKTKPREEQYNSTYRVVSVLTVLHQDWLNGKEYKCKVSNKALPAPIEKTISKAKGQPREPQVYTLPPSRDELTKNQVSLTCLVKGFYPSDIAVEWESNGQPENNYKTTPPVLDSDGSFFLYSKLTVDKSRWQQGNVFSCSVMHEALHNHYTQKSLSLSPGK

SEQ ID NO: 5 - protein, 740 aa, Artificial Sequence
  QD3745
MEFGLSWLFLVAILKGVQCDIVMTQSPDSLAVSLGERATINCKSSQSLLNSGNQKNYLAWYQQKPGQPPKLLIYGASTRESGVPDRFTGSGSGTDFTLTISSLQAEDVAVYYCQNDHSYPFTFGQGTKLEIKRTVAAPSVFIFPPSDEQLKSGTASVVCLLNNFYPREAKVQWKVDNALQSGNSQESVTEQDSKDSTYSLSSTLTLSKADYEKHKVYACEVTHQGLSSPVTKSFNRGECGGGGSGGGGSEVQLLESGGGLVQPGGSLKLSCAASGFTFNTYAMNWVRQAPGKGLEWVARIRSKYNNYATYYADSVKDRFTISRDDSKNTAYLQMNNLKTEDTAVYYCVRHGNFGNSYVSWFAYWGQGTLVTVSSGGGGSGGGGSGGGGSELVVTQEPSLTVSPGGTVTLTCRSSTGAVTTSNYANWVQQKPGQAPRGLIGGTNKRAPGTPARFSGSLLGGKAALTLSGVQPEDEAEYYCALWYSNLWVFGGGTKLTVLGGGGSESKYGPPCPPCPAPEFLGGPSVFLFPPKPKDTLMISRTPEVTCVVVDVSQEDPEVQFNWYVDGVEVHNAKTKPREEQFNSTYRVVSVLTVLHQDWLNGKEYKCKVSNKGLPSSIEKTISKAKGQPREPQVYTLPPSQEEMTKNQVSLWCLVKGFYPSDIAVEWESNGQPENNYKTTPPVLDSDGSFFLYSRLTVDKSRWQEGNVFSCSVMHEALHNHYTQKSLSLSLGGSSHHHHHH

SEQ ID NO: 6 - protein, 478 aa, Artificial Sequence
  QD3749
MEFGLSWLFLVAILKGVQCDIVMTQSPDSLAVSLGERATINCKSSQSLLNSGNQKNYLAWYQQKPGQPPKLLIYGASTRESGVPDRFTGSGSGTDFTLTISSLQAEDVAVYYCQNDHSYPFTFGQGTKLEIKRTVAAPSVFIFPPSDEQLKSGTASVVCLLNNFYPREAKVQWKVDNALQSGNSQESVTEQDSKDSTYSLSSTLTLSKADYEKHKVYACEVTHQGLSSPVTKSFNRGECESKYGPPCPPCPAPEFLGGPSVFLFPPKPKDTLMISRTPEVTCVVVDVSQEDPEVQFNWYVDGVEVHNAKTKPREEQFNSTYRVVSVLTVLHQDWLNGKEYKCKVSNKGLPSSIEKTISKAKGQPREPQVYTLPPSQEEMTKNQVSLSCAVKGFYPSDIAVEWESNGQPENNYKTTPPVLDSDGSFFLVSRLTVDKSRWQEGNVFSCSVMHEALHNHYTQKSLSLSLGGSSDYKDDDDK

SEQ ID NO: 7 - protein, 242 aa, Artificial Sequence
  QD3746
MEFGLSWLFLVAILKGVQCQVQLVQSGAEVKKPGASVKVSCKASGYTFTSYIMHWVRQAPGQGLEWMGYINPYNDGTKYNEKFKGRVTMTRDTSTSTVYMELSSLRSEDTAVYYCARLGFTTRNAMDYWGQGTLVTVSSASTKGPSVFPLAPSSKSTSGGTAALGCLVKDYFPEPVTVSWNSGALTSGVHTFPAVLQSSGLYSLSSVVTVPSSSLGTQTYICNVNHKPSNTKVDKKVEPKSC

SEQ ID NO: 8 - protein, 740 aa, Artificial Sequence
  QD908
MEFGLSWLFLVAILKGVQCDIVMTQSPDSLAVSLGERATINCKSSQSLLNSGNQKNYLAWYQQKPGQPPKLLIYGASTRESGVPDRFTGSGSGTDFTLTISSLQAEDVAVYYCQNDHSYPFTFGQGTKLEIKRTVAAPSVFIFPPSDEQLKSGTASVVCLLNNFYPREAKVQWKVDNALQSGNSQESVTEQDSKDSTYSLSSTLTLSKADYEKHKVYACEVTHQGLSSPVTKSFNRGECGGGGSGGGGSEVQLLESGGGLVQPGGSLKLSCAASGFTFNTYAMNWVRQAPGKGLEWVARIRSKYNNYETYYADSVKDRFTISRDDSKNTAYLQMNNLKTEDTAVYYCVRHGNFGNSYVSWFAYWGQGTLVTVSSGGGGSGGGGSGGGGSELVVTQEPSLTVSPGGTVTLTCRSSTGAVTTSNYANWVQQKPGQAPRGLIGGTNLRAPGTPARFSGSLLGGKAALTLSGVQPEDEAEYYCALWRSGGWVFGGGTKLTVLGGGGSESKYGPPCPPCPAPEFLGGPSVFLFPPKPKDTLMISRTPEVTCVVVDVSQEDPEVQFNWYVDGVEVHNAKTKPREEQFNSTYRVVSVLTVLHQDWLNGKEYKCKVSNKGLPSSIEKTISKAKGQPREPQVYTLPPSQEEMTKNQVSLWCLVKGFYPSDIAVEWESNGQPENNYKTTPPVLDSDGSFFLYSRLTVDKSRWQEGNVFSCSVMHEALHNHYTQKSLSLSLGGSSHHHHHH

SEQ ID NO: 9 - protein, 740 aa, Artificial Sequence
  QD909
MEFGLSWLFLVAILKGVQCDIVMTQSPDSLAVSLGERATINCKSSQSLLNSGNQKNYLAWYQQKPGQPPKLLIYGASTRESGVPDRFTGSGSGTDFTLTISSLQAEDVAVYYCQNDHSYPFTFGQGTKLEIKRTVAAPSVFIFPPSDEQLKSGTASVVCLLNNFYPREAKVQWKVDNALQSGNSQESVTEQDSKDSTYSLSSTLTLSKADYEKHKVYACEVTHQGLSSPVTKSFNRGECGGGGSGGGGSEVQLLESGGGLVQPGGSLKLSCAASGFTFNTYAMNWVRQAPGKGLEWVARIRSKYNNYETYYADSVKDRFTISRDDSKNTAYLQMNNLKTEDTAVYYCVRHSNFGNGYVSWFAYWGQGTLVTVSSGGGGSGGGGSGGGGSELVVTQEPSLTVSPGGTVTLTCRSSTGAVTTSNYANWVQQKPGQAPRGLIGGTNLRAPGTPARFSGSLLGGKAALTLSGVQPEDEAEYYCALWNKGGWVFGGGTKLTVLGGGGSESKYGPPCPPCPAPEFLGGPSVFLFPPKPKDTLMISRTPEVTCVVVDVSQEDPEVQFNWYVDGVEVHNAKTKPREEQFNSTYRVVSVLTVLHQDWLNGKEYKCKVSNKGLPSSIEKTISKAKGQPREPQVYTLPPSQEEMTKNQVSLWCLVKGFYPSDIAVEWESNGQPENNYKTTPPVLDSDGSFFLYSRLTVDKSRWQEGNVFSCSVMHEALHNHYTQKSLSLSLGGSSHHHHHH

SEQ ID NO: 10 - protein, 740 aa, Artificial Sequence
  QD910
MEFGLSWLFLVAILKGVQCDIVMTQSPDSLAVSLGERATINCKSSQSLLNSGNQKNYLAWYQQKPGQPPKLLIYGASTRESGVPDRFTGSGSGTDFTLTISSLQAEDVAVYYCQNDHSYPFTFGQGTKLEIKRTVAAPSVFIFPPSDEQLKSGTASVVCLLNNFYPREAKVQWKVDNALQSGNSQESVTEQDSKDSTYSLSSTLTLSKADYEKHKVYACEVTHQGLSSPVTKSFNRGECGGGGSGGGGSEVQLLESGGGLVQPGGSLKLSCAASGFTFNTYAMNWVRQAPGKGLEWVARIRSKYNNYETYYADSVKDRFTISRDDSKNTAYLQMNNLKTEDTAVYYCVRHSNFGNGYVSWFAYWGQGTLVTVSSGGGGSGGGGSGGGGSELVVTQEPSLTVSPGGTVTLTCRSSTGAVTTSNYANWVQQKPGQAPRGLIGGTWLRAPGTPARFSGSLLGGKAALTLSGVQPEDEAEYYCALWNSGGWVFGGGTKLTVLGGGGSESKYGPPCPPCPAPEFLGGPSVFLFPPKPKDTLMISRTPEVTCVVVDVSQEDPEVQFNWYVDGVEVHNAKTKPREEQFNSTYRVVSVLTVLHQDWLNGKEYKCKVSNKGLPSSIEKTISKAKGQPREPQVYTLPPSQEEMTKNQVSLWCLVKGFYPSDIAVEWESNGQPENNYKTTPPVLDSDGSFFLYSRLTVDKSRWQEGNVFSCSVMHEALHNHYTQKSLSLSLGGSSHHHHHH

SEQ ID NO: 11 - protein, 636 aa, Artificial Sequence
  QD3723
MEFGLSWLFLVAILKGVQCQVQLVQSGAEVKKPGASVKVSCKASGYTFTSYIMHWVRQAPGQGLEWMGYINPYNDGTKYNEKFKGRVTMTRDTSTSTVYMELSSLRSEDTAVYYCARLGFTTRNAMDYWGQGTLVTVSSASTKGPSVFPLAPSSKSTSGGTAALGCLVKDYFPEPVTVSWNSGALTSGVHTFPAVLQSSGLYSLSSVVTVPSSSLGTQTYICNVNHKPSNTKVDKKVEPKSCGGGGSGGGGSGGGGSEVQLLESGGGLVQPGGSLKLSCAASGFTFNTYAMNWVRQAPGKGLEWVARIRSKYNNYATYYADSVKDRFTISRDDSKNTAYLQMNNLKTEDTAVYYCVRHGNFGNSYVSWFAYWGQGTLVTVSSGGGGSGGGGSGGGGSESKYGPPCPPCPAPEFLGGPSVFLFPPKPKDTLMISRTPEVTCVVVDVSQEDPEVQFNWYVDGVEVHNAKTKPREEQFNSTYRVVSVLTVLHQDWLNGKEYKCKVSNKGLPSSIEKTISKAKGQPREPQVYTLPPSQEEMTKNQVSLSCAVKGFYPSDIAVEWESNGQPENNYKTTPPVLDSDGSFFLVSRLTVDKSRWQEGNVFSCSVMHEALHNHYTQKSLSLSLGGSSDYKDDDDK

SEQ ID NO: 12 - protein, 618 aa, Artificial Sequence
  QD3724
MEFGLSWLFLVAILKGVQCQVQLVQSGAEVKKPGASVKVSCKASGYTFTSYIMHWVRQAPGQGLEWMGYINPYNDGTKYNEKFKGRVTMTRDTSTSTVYMELSSLRSEDTAVYYCARLGFTTRNAMDYWGQGTLVTVSSASTKGPSVFPLAPSSKSTSGGTAALGCLVKDYFPEPVTVSWNSGALTSGVHTFPAVLQSSGLYSLSSVVTVPSSSLGTQTYICNVNHKPSNTKVDKKVEPKSCGGGGSGGGGSGGGGSELVVTQEPSLTVSPGGTVTLTCRSSTGAVTTSNYANWVQQKPGQAPRGLIGGTNKRAPGTPARFSGSLLGGKAALTLSGVQPEDEAEYYCALWYSNLWVFGGGTKLTVLGGGGSGGGGSGGGGSESKYGPPCPPCPAPEFLGGPSVFLFPPKPKDTLMISRTPEVTCVVVDVSQEDPEVQFNWYVDGVEVHNAKTKPREEQFNSTYRVVSVLTVLHQDWLNGKEYKCKVSNKGLPSSIEKTISKAKGQPREPQVYTLPPSQEEMTKNQVSLWCLVKGFYPSDIAVEWESNGQPENNYKTTPPVLDSDGSFFLYSRLTVDKSRWQEGNVFSCSVMHEALHNHYTQKSLSLSLGGSSHHHHHH

SEQ ID NO: 13 - protein, 242 aa, Artificial Sequence
  QDl461
MDMRVPAQLLGLLLLWFPGSRCDIVMTQSPDSLAVSLGERATINCKSSQSLLNSGNQKNYLAWYQQKPGQPPKLLIYGASTRESGVPDRFTGSGSGTDFTLTISSLQAEDVAVYYCQNDHSYPFTFGQGTKLEIKRTVAAPSVFIFPPSDEQLKSGTASVVCLLNNFYPREAKVQWKVDNALQSGNSQESVTEQDSKDSTYSLSSTLTLSKADYEKHKVYACEVTHQGLSSPVTKSFNRGEC

SEQ ID NO: 14 - protein, 743 aa, Artificial Sequence
  QD3744
MEFGLSWLFLVAILKGVQCQVQLVQSGAEVKKPGASVKVSCKASGYTFTSYIMHWVRQAPGQGLEWMGYINPYNDGTKYNEKFKGRVTMTRDTSTSTVYMELSSLRSEDTAVYYCARLGFTTRNAMDYWGQGTLVTVSSASTKGPSVFPLAPSSKSTSGGTAALGCLVKDYFPEPVTVSWNSGALTSGVHTFPAVLQSSGLYSLSSVVTVPSSSLGTQTYICNVNHKPSNTKVDKKVEPKSCGGGGSGGGGSEVQLLESGGGLVQPGGSLKLSCAASGFTFNTYAMNWVRQAPGKGLEWVARIRSKYNNYATYYADSVKDRFTISRDDSKNTAYLQMNNLKTEDTAVYYCVRHGNFGNSYVSWFAYWGQGTLVTVSSGGGGSGGGGSGGGGSELVVTQEPSLTVSPGGTVTLTCRSSTGAVTTSNYANWVQQKPGQAPRGLIGGTNKRAPGTPARFSGSLLGGKAALTLSGVQPEDEAEYYCALWYSNLWVFGGGTKLTVLGGGGSESKYGPPCPPCPAPEFLGGPSVFLFPPKPKDTLMISRTPEVTCVVVDVSQEDPEVQFNWYVDGVEVHNAKTKPREEQFNSTYRVVSVLTVLHQDWLNGKEYKCKVSNKGLPSSIEKTISKAKGQPREPQVYTLPPSQEEMTKNQVSLWCLVKGFYPSDIAVEWESNGQPENNYKTTPPVLDSDGSFFLYSRLTVDKSRWQEGNVFSCSVMHEALHNHYTQKSLSLSLGGSSHHHHHH

SEQ ID NO: 15 - protein, 481 aa, Artificial Sequence
  QD3748
MEFGLSWLFLVAILKGVQCQVQLVQSGAEVKKPGASVKVSCKASGYTFTSYIMHWVRQAPGQGLEWMGYINPYNDGTKYNEKFKGRVTMTRDTSTSTVYMELSSLRSEDTAVYYCARLGFTTRNAMDYWGQGTLVTVSSASTKGPSVFPLAPSSKSTSGGTAALGCLVKDYFPEPVTVSWNSGALTSGVHTFPAVLQSSGLYSLSSVVTVPSSSLGTQTYICNVNHKPSNTKVDKKVEPKSCESKYGPPCPPCPAPEFLGGPSVFLFPPKPKDTLMISRTPEVTCVVVDVSQEDPEVQFNWYVDGVEVHNAKTKPREEQFNSTYRVVSVLTVLHQDWLNGKEYKCKVSNKGLPSSIEKTISKAKGQPREPQVYTLPPSQEEMTKNQVSLSCAVKGFYPSDIAVEWESNGQPENNYKTTPPVLDSDGSFFLVSRLTVDKSRWQEGNVFSCSVMHEALHNHYTQKSLSLSLGGSSDYKDDDDK

SEQ ID NO: 16 - protein, 990 aa, Artificial Sequence
  QD3693
QVQLVQSGAEVKKPGASVKVSCKASGYTFTGYYMHWVRQAPGQCLEWMGWINPNSGGTKYAQKFQGRVTMTRDTSISTAYMELSRLRSDDTAVYYCARDRITVAGTYYYYGMDVWGQGTTVTVSSGGGGSGGGGSGGGGSDIQMTQSPSSVSASVGDRVTITCRASQGVNNWLAWYQQKPGKAPKLLIYTASSLQSGVPSRFSGSGSGTDFTLTIRSLQPEDFATYYCQQANSFPITFGCGTRLEIKSGGGGSEVQLVESGGGLVQPGGSLKLSCAASGFTFNKYAMNWVRQAPGKGLEWVARIRSKYNNYATYYADSVKDRFTISRDDSKNTAYLQMNNLKTEDTAVYYCVRHGNFGNSYISYWAYWGQGTLVTVSSGGGGSGGGGSGGGGSQTVVTQEPSLTVSPGGTVTLTCGSSTGAVTSGNYPNWVQQKPGQAPRGLIGGTKFLAPGTPARFSGSLLGGKAALTLSGVQPEDEAEYYCVLWYSNRWVFGGGTKLTVLGGGGDKTHTCPPCPAPELLGGPSVFLFPPKPKDTLMISRTPEVTCVVVDVSHEDPEVKFNWYVDGVEVHNAKTKPCEEQYGSTYRCVSVLTVLHQDWLNGKEYKCKVSNKALPAPIEKTISKAKGQPREPQVYTLPPSREEMTKNQVSLTCLVKGFYPSDIAVEWESNGQPENNYKTTPPVLDSDGSFFLYSKLTVDKSRWQQGNVFSCSVMHEALHNHYTQKSLSLSPGKGGGGSGGGGSGGGGSGGGGSGGGGSGGGGSDKTHTCPPCPAPELLGGPSVFLFPPKPKDTLMISRTPEVTCVVVDVSHEDPEVKFNWYVDGVEVHNAKTKPCEEQYGSTYRCVSVLTVLHQDWLNGKEYKCKVSNKALPAPIEKTISKAKGQPREPQVYTLPPSREEMTKNQVSLTCLVKGFYPSDIAVEWESNGQPENNYKTTPPVLDSDGSFFLYSKLTVDKSRWQQGNVFSCSVMHEALHNHYTQKSLSLSPGK

SEQ ID NO: 17 - protein, 692 aa, Artificial Sequence
  QD0899
MEFGLSWLFLVAILKGVQCDIVMTQSPDSLAVSLGERATINCKSSQSLLNSGNQKNYLAWYQQKPGQPPKLLIYGASTRESGVPDRFTGSGSGTDFTLTISSLQAEDVAVYYCQNDHSYPFTFGQGTKLEIKRTVAAPSVFIFPPSDEQLKSGTASVVCLLNNFYPREAKVQWKVDNALQSGNSQESVTEQDSKDSTYSLSSTLTLSKADYEKHKVYACEVTHQGLSSPVTKSFNRGECGGGGSGGGGSITCPPPMSVEHADIWVKSYSLYSRERYICNSGFKRKAGTCSLTECVLNKATNVAHWTTPSLKCIRSGGSGGGGSGGGSGGGGSLQNWVNVISDLKKIEDLIQSMHIDATLYTESDVHPSCKVTAMKCFLLELQVISCESGDASIHDTVENLIILANNSLSSNGNVTESGCKECEELEEKNIKEFLQSFVHIVQMFINTSGGGGSESKYGPPCPPCPAPEFLGGPSVFLFPPKPKDTLMISRTPEVTCVVVDVSQEDPEVQFNWYVDGVEVHNAKTKPREEQFNSTYRVVSVLTVLHQDWLNGKEYKCKVSNKGLPSSIEKTISKAKGQPREPQVYTLPPSQEEMTKNQVSLSCAVKGFYPSDIAVEWESNGQPENNYKTTPPVLDSDGSFFLVSRLTVDKSRWQEGNVFSCSVMHEALHNHYTQKSLSLSLGGSSDYKDDDDK

SEQ ID NO: 18 - protein, 697 aa, Artificial Sequence
  QD0900
MEFGLSWLFLVAILKGVQCDIVMTQSPDSLAVSLGERATINCKSSQSLLNSGNQKNYLAWYQQKPGQPPKLLIYGASTRESGVPDRFTGSGSGTDFTLTISSLQAEDVAVYYCQNDHSYPFTFGQGTKLEIKRTVAAPSVFIFPPSDEQLKSGTASVVCLLNNFYPREAKVQWKVDNALQSGNSQESVTEQDSKDSTYSLSSTLTLSKADYEKHKVYACEVTHQGLSSPVTKSFNRGECGGGGSGGGGNWVNVISDLKKIEDLIQSMHIDATLYTESDVHPSCKVTAMKCFLLELQVISCESGDASIHDTVENLIILANNSLSSNGNVTESGCKECEELEEKNIKEFLQSFVHIVQMFINTSSGGGSGGGGSGGGGSGGGGSGGGSGGITCPPPMSVEHADIWVKSYSLYSRERYICNSGFKRKAGTCSLTECVLNKATNVAHWTTPSLKCIRGGGGSESKYGPPCPPCPAPEFLGGPSVFLFPPKPKDTLMISRTPEVTCVVVDVSQEDPEVQFNWYVDGVEVHNAKTKPREEQFNSTYRVVSVLTVLHQDWLNGKEYKCKVSNKGLPSSIEKTISKAKGQPREPQVYTLPPSQEEMTKNQVSLSCAVKGFYPSDIAVEWESNGQPENNYKTTPPVLDSDGSFFLVSRLTVDKSRWQEGNVFSCSVMHEALHNHYTQKSLSLSLGGSSDYKDDDDK

SEQ ID NO: 19 - protein, 740 aa, Artificial Sequence
  QD0901
MEFGLSWLFLVAILKGVQCDIVMTQSPDSLAVSLGERATINCKSSQSLLNSGNQKNYLAWYQQKPGQPPKLLIYGASTRESGVPDRFTGSGSGTDFTLTISSLQAEDVAVYYCQNDHSYPFTFGQGTKLEIKRTVAAPSVFIFPPSDEQLKSGTASVVCLLNNFYPREAKVQWKVDNALQSGNSQESVTEQDSKDSTYSLSSTLTLSKADYEKHKVYACEVTHQGLSSPVTKSFNRGECGGGGSGGGGSELVVTQEPSLTVSPGGTVTLTCRSSTGAVTTSNYANWVQQKPGQAPRGLIGGTNKRAPGTPARFSGSLLGGKAALTLSGVQPEDEAEYYCALWYSNLWVFGGGTKLTVLGGGGSGGGGSGGGGSEVQLLESGGGLVQPGGSLKLSCAASGFTFNTYAMNWVRQAPGKGLEWVARIRSKYNNYATYYADSVKDRFTISRDDSKNTAYLQMNNLKTEDTAVYYCVRHGNFGNSYVSWFAYWGQGTLVTVSSGGGGSESKYGPPCPPCPAPEFLGGPSVFLFPPKPKDTLMISRTPEVTCVVVDVSQEDPEVQFNWYVDGVEVHNAKTKPREEQFNSTYRVVSVLTVLHQDWLNGKEYKCKVSNKGLPSSIEKTISKAKGQPREPQVYTLPPSQEEMTKNQVSLWCLVKGFYPSDIAVEWESNGQPENNYKTTPPVLDSDGSFFLYSRLTVDKSRWQEGNVFSCSVMHEALHNHYTQKSLSLSLGGSSHHHHHH

SEQ ID NO: 20 - protein, 731 aa, Artificial Sequence
  QD3667
MEFGLSWLFLVAILKGVQCDIVMTQSPDSLAVSLGERATINCKSSQSLLNSGNQKNYLAWYQQKPGQPPKLLIYGASTRESGVPDRFTGSGSGTDFTLTISSLQAEDVAVYYCQNDHSYPFTFGQGTKLEIKGGGGSGGGGSGGGGSQVQLVQSGAEVKKPGASVKVSCKASGYTFTSYIMHWVRQAPGQGLEWMGYINPYNDGTKYNEKFKGRVTMTRDTSTSTVYMELSSLRSEDTAVYYCARLGFTTRNAMDYWGQGTLVTVSSGGGGSGGGGSGGGGSNWVNVISDLKKIEDLIQSMHIDATLYTESDVHPSCKVTAMKCFLLELQVISCESGDASIHDTVENLIILANNSLSSNGNVTESGCKECEELEEKNIKEFLQSFVHIVQMFINTSSGGGSGGGGSGGGGSGGGGSGGGSGGITCPPPMSVEHADIWVKSYSLYSRERYICNSGFKRKAGTCSLTECVLNKATNVAHWTTPSLKCIRGGGGSESKYGPPCPPCPAPEFLGGPSVFLFPPKPKDTLMISRTPEVTCVVVDVSQEDPEVQFNWYVDGVEVHNAKTKPREEQFNSTYRVVSVLTVLHQDWLNGKEYKCKVSNKGLPSSIEKTISKAKGQPREPQVYTLPPSQEEMTKNQVSLSCAVKGFYPSDIAVEWESNGQPENNYKTTPPVLDSDGSFFLVSRLTVDKSRWQEGNVFSCSVMHEALHNHYTQKSLSLSLGGSSDYKDDDDK

SEQ ID NO: 21 - protein, 763 aa, Artificial Sequence
  QD3668
MEFGLSWLFLVAILKGVQCDIVMTQSPDSLAVSLGERATINCKSSQSLLNSGNQKNYLAWYQQKPGQPPKLLIYGASTRESGVPDRFTGSGSGTDFTLTISSLQAEDVAVYYCQNDHSYPFTFGQGTKLEIKGGGGSGGGGSGGGGSQVQLVQSGAEVKKPGASVKVSCKASGYTFTSYIMHWVRQAPGQGLEWMGYINPYNDGTKYNEKFKGRVTMTRDTSTSTVYMELSSLRSEDTAVYYCARLGFTTRNAMDYWGQGTLVTVSSGGGGSEVQLLESGGGLVQPGGSLKLSCAASGFTFNTYAMNWVRQAPGKGLEWVARIRSKYNNYATYYADSVKDRFTISRDDSKNTAYLQMNNLKTEDTAVYYCVRHGNFGNSYVSWFAYWGQGTLVTVSSGGGGSGGGGSGGGGSELVVTQEPSLTVSPGGTVTLTCRSSTGAVTTSNYANWVQQKPGQAPRGLIGGTNKRAPGTPARFSGSLLGGKAALTLSGVQPEDEAEYYCALWYSNLWVFGGGTKLTVLGGGGSESKYGPPCPPCPAPEFLGGPSVFLFPPKPKDTLMISRTPEVTCVVVDVSQEDPEVQFNWYVDGVEVHNAKTKPREEQFNSTYRVVSVLTVLHQDWLNGKEYKCKVSNKGLPSSIEKTISKAKGQPREPQVYTLPPSQEEMTKNQVSLWCLVKGFYPSDIAVEWESNGQPENNYKTTPPVLDSDGSFFLYSRLTVDKSRWQEGNVFSCSVMHEALHNHYTQKSLSLSLGGSSHHHHHH

SEQ ID NO: 22 - protein, 725 aa, Artificial Sequence
  QD0902
MEFGLSWLFLVAILKGVQCDIVMTQSPDSLAVSLGERATINCKSSQSLLNSGNQKNYLAWYQQKPGQPPKLLIYGASTRESGVPDRFTGSGSGTDFTLTISSLQAEDVAVYYCQNDHSYPFTFGQGTKLEIKGGGGSGGGGSGGGGSQVQLVQSGAEVKKPGASVKVSCKASGYTFTSYIMHWVRQAPGQGLEWMGYINPYNDGTKYNEKFKGRVTMTRDTSTSTVYMELSSLRSEDTAVYYCARLGFTTRNAMDYWGQGTLVTVSSGGGGSGGGGSGGGGSITCPPPMSVEHADIWVKSYSLYSRERYICNSGFKRKAGTCSLTECVLNKATNVAHWTTPSLKCIRSGGSGGGGSGGGSGGGGSLQNWVNVISDLKKIEDLIQSMHIDATLYTESDVHPSCKVTAMKCFLLELQVISCESGDASIHDTVENLIILANNSLSSNGNVTESGCKECEELEEKNIKEFLQSFVHIVQMFINTSGGGGSESKYGPPCPPCPAPEFLGGPSVFLFPPKPKDTLMISRTPEVTCVVVDVSQEDPEVQFNWYVDGVEVHNAKTKPREEQFNSTYRVVSVLTVLHQDWLNGKEYKCKVSNKGLPSSIEKTISKAKGQPREPQVYTLPPSQEEMTKNQVSLSCAVKGFYPSDIAVEWESNGQPENNYKTTPPVLDSDGSFFLVSRLTVDKSRWQEGNVFSCSVMHEALHNHYTQKSLSLSLGGSSDYKDDDDK

SEQ ID NO: 23 - protein, 763 aa, Artificial Sequence
  QD0903
MEFGLSWLFLVAILKGVQCDIVMTQSPDSLAVSLGERATINCKSSQSLLNSGNQKNYLAWYQQKPGQPPKLLIYGASTRESGVPDRFTGSGSGTDFTLTISSLQAEDVAVYYCQNDHSYPFTFGQGTKLEIKGGGGSGGGGSGGGGSQVQLVQSGAEVKKPGASVKVSCKASGYTFTSYIMHWVRQAPGQGLEWMGYINPYNDGTKYNEKFKGRVTMTRDTSTSTVYMELSSLRSEDTAVYYCARLGFTTRNAMDYWGQGTLVTVSSGGGGSELVVTQEPSLTVSPGGTVTLTCRSSTGAVTTSNYANWVQQKPGQAPRGLIGGTNKRAPGTPARFSGSLLGGKAALTLSGVQPEDEAEYYCALWYSNLWVFGGGTKLTVLGGGGSGGGGSGGGGSEVQLLESGGGLVQPGGSLKLSCAASGFTFNTYAMNWVRQAPGKGLEWVARIRSKYNNYATYYADSVKDRFTISRDDSKNTAYLQMNNLKTEDTAVYYCVRHGNFGNSYVSWFAYWGQGTLVTVSSGGGGSESKYGPPCPPCPAPEFLGGPSVFLFPPKPKDTLMISRTPEVTCVVVDVSQEDPEVQFNWYVDGVEVHNAKTKPREEQFNSTYRVVSVLTVLHQDWLNGKEYKCKVSNKGLPSSIEKTISKAKGQPREPQVYTLPPSQEEMTKNQVSLWCLVKGFYPSDIAVEWESNGQPENNYKTTPPVLDSDGSFFLYSRLTVDKSRWQEGNVFSCSVMHEALHNHYTQKSLSLSLGGSSHHHHHH

SEQ ID NO: 24 - protein, 731 aa, Artificial Sequence
  QD0904
MEFGLSWLFLVAILKGVQCQVQLVQSGAEVKKPGASVKVSCKASGYTFTSYIMHWVRQAPGQGLEWMGYINPYNDGTKYNEKFKGRVTMTRDTSTSTVYMELSSLRSEDTAVYYCARLGFTTRNAMDYWGQGTLVTVSSGGGGSGGGGSGGGGSDIVMTQSPDSLAVSLGERATINCKSSQSLLNSGNQKNYLAWYQQKPGQPPKLLIYGASTRESGVPDRFTGSGSGTDFTLTISSLQAEDVAVYYCQNDHSYPFTFGQGTKLEIKGGGGSGGGGSGGGGSNWVNVISDLKKIEDLIQSMHIDATLYTESDVHPSCKVTAMKCFLLELQVISCESGDASIHDTVENLIILANNSLSSNGNVTESGCKECEELEEKNIKEFLQSFVHIVQMFINTSSGGGSGGGGSGGGGSGGGGSGGGSGGITCPPPMSVEHADIWVKSYSLYSRERYICNSGFKRKAGTCSLTECVLNKATNVAHWTTPSLKCIRGGGGSESKYGPPCPPCPAPEFLGGPSVFLFPPKPKDTLMISRTPEVTCVVVDVSQEDPEVQFNWYVDGVEVHNAKTKPREEQFNSTYRVVSVLTVLHQDWLNGKEYKCKVSNKGLPSSIEKTISKAKGQPREPQVYTLPPSQEEMTKNQVSLSCAVKGFYPSDIAVEWESNGQPENNYKTTPPVLDSDGSFFLVSRLTVDKSRWQEGNVFSCSVMHEALHNHYTQKSLSLSLGGSSDYKDDDDK

SEQ ID NO: 25 - protein, 763 aa, Artificial Sequence
  QD0905
MEFGLSWLFLVAILKGVQCQVQLVQSGAEVKKPGASVKVSCKASGYTFTSYIMHWVRQAPGQGLEWMGYINPYNDGTKYNEKFKGRVTMTRDTSTSTVYMELSSLRSEDTAVYYCARLGFTTRNAMDYWGQGTLVTVSSGGGGSGGGGSGGGGSDIVMTQSPDSLAVSLGERATINCKSSQSLLNSGNQKNYLAWYQQKPGQPPKLLIYGASTRESGVPDRFTGSGSGTDFTLTISSLQAEDVAVYYCQNDHSYPFTFGQGTKLEIKGGGGSEVQLLESGGGLVQPGGSLKLSCAASGFTFNTYAMNWVRQAPGKGLEWVARIRSKYNNYATYYADSVKDRFTISRDDSKNTAYLQMNNLKTEDTAVYYCVRHGNFGNSYVSWFAYWGQGTLVTVSSGGGGSGGGGSGGGGSELVVTQEPSLTVSPGGTVTLTCRSSTGAVTTSNYANWVQQKPGQAPRGLIGGTNKRAPGTPARFSGSLLGGKAALTLSGVQPEDEAEYYCALWYSNLWVFGGGTKLTVLGGGGSESKYGPPCPPCPAPEFLGGPSVFLFPPKPKDTLMISRTPEVTCVVVDVSQEDPEVQFNWYVDGVEVHNAKTKPREEQFNSTYRVVSVLTVLHQDWLNGKEYKCKVSNKGLPSSIEKTISKAKGQPREPQVYTLPPSQEEMTKNQVSLWCLVKGFYPSDIAVEWESNGQPENNYKTTPPVLDSDGSFFLYSRLTVDKSRWQEGNVFSCSVMHEALHNHYTQKSLSLSLGGSSHHHHHH

SEQ ID NO: 26 - protein, 725 aa, Artificial Sequence
  QD0906
MEFGLSWLFLVAILKGVQCQVQLVQSGAEVKKPGASVKVSCKASGYTFTSYIMHWVRQAPGQGLEWMGYINPYNDGTKYNEKFKGRVTMTRDTSTSTVYMELSSLRSEDTAVYYCARLGFTTRNAMDYWGQGTLVTVSSGGGGSGGGGSGGGGSDIVMTQSPDSLAVSLGERATINCKSSQSLLNSGNQKNYLAWYQQKPGQPPKLLIYGASTRESGVPDRFTGSGSGTDFTLTISSLQAEDVAVYYCQNDHSYPFTFGQGTKLEIKGGGGSGGGGSGGGGSITCPPPMSVEHADIWVKSYSLYSRERYICNSGFKRKAGTCSLTECVLNKATNVAHWTTPSLKCIRSGGSGGGGSGGGSGGGGSLQNWVNVISDLKKIEDLIQSMHIDATLYTESDVHPSCKVTAMKCFLLELQVISCESGDASIHDTVENLIILANNSLSSNGNVTESGCKECEELEEKNIKEFLQSFVHIVQMFINTSGGGGSESKYGPPCPPCPAPEFLGGPSVFLFPPKPKDTLMISRTPEVTCVVVDVSQEDPEVQFNWYVDGVEVHNAKTKPREEQFNSTYRVVSVLTVLHQDWLNGKEYKCKVSNKGLPSSIEKTISKAKGQPREPQVYTLPPSQEEMTKNQVSLSCAVKGFYPSDIAVEWESNGQPENNYKTTPPVLDSDGSFFLVSRLTVDKSRWQEGNVFSCSVMHEALHNHYTQKSLSLSLGGSSDYKDDDDK

SEQ ID NO: 27 - protein, 763 aa, Artificial Sequence
  QD0907
MEFGLSWLFLVAILKGVQCQVQLVQSGAEVKKPGASVKVSCKASGYTFTSYIMHWVRQAPGQGLEWMGYINPYNDGTKYNEKFKGRVTMTRDTSTSTVYMELSSLRSEDTAVYYCARLGFTTRNAMDYWGQGTLVTVSSGGGGSGGGGSGGGGSDIVMTQSPDSLAVSLGERATINCKSSQSLLNSGNQKNYLAWYQQKPGQPPKLLIYGASTRESGVPDRFTGSGSGTDFTLTISSLQAEDVAVYYCQNDHSYPFTFGQGTKLEIKGGGGSELVVTQEPSLTVSPGGTVTLTCRSSTGAVTTSNYANWVQQKPGQAPRGLIGGTNKRAPGTPARFSGSLLGGKAALTLSGVQPEDEAEYYCALWYSNLWVFGGGTKLTVLGGGGSGGGGSGGGGSEVQLLESGGGLVQPGGSLKLSCAASGFTFNTYAMNWVRQAPGKGLEWVARIRSKYNNYATYYADSVKDRFTISRDDSKNTAYLQMNNLKTEDTAVYYCVRHGNFGNSYVSWFAYWGQGTLVTVSSGGGGSESKYGPPCPPCPAPEFLGGPSVFLFPPKPKDTLMISRTPEVTCVVVDVSQEDPEVQFNWYVDGVEVHNAKTKPREEQFNSTYRVVSVLTVLHQDWLNGKEYKCKVSNKGLPSSIEKTISKAKGQPREPQVYTLPPSQEEMTKNQVSLWCLVKGFYPSDIAVEWESNGQPENNYKTTPPVLDSDGSFFLYSRLTVDKSRWQEGNVFSCSVMHEALHNHYTQKSLSLSLGGSSHHHHHH

SEQ ID NO: 28 - protein, 721 aa, Artificial Sequence
  QD0728
MEFGLSWLFLVAILKGVQCDIVMTQSPDSLAVSLGERATINCKSSQSLLNSGNQKNYLAWYQQKPGQPPKLLIYGASTRESGVPDRFTGSGSGTDFTLTISSLQAEDVAVYYCQNDHSYPFTFGQGTKLEIKGGGGSGGGGSGGGGSQVQLVQSGAEVKKPGASVKVSCKASGYTFTSYIMHWVRQAPGQGLEWMGYINPYNDGTKYNEKFKGRVTMTRDTSTSTVYMELSSLRSEDTAVYYCARLGFTTRNAMDYWGQGTLVTVSSGGGGSGGGGSGGGGSNWVNVISDLKKIEDLIQSMHIDATLYTESDVHPSCKVTAMKCFLLELQVISCESGDASIHDTVENLIILANNSLSSNGNVTESGCKECEELEEKNIKEFLQSFVHIVQMFINTSSGGGSGGGGSGGGGSGGGGSGGGSGGITCPPPMSVEHADIWVKSYSLYSRERYICNSGFKRKAGTCSLTECVLNKATNVAHWTTPSLKCIRGGGGSESKYGPPCPPCPAPEFLGGPSVFLFPPKPKDTLMISRTPEVTCVVVDVSQEDPEVQFNWYVDGVEVHNAKTKPREEQFNSTYRVVSVLTVLHQDWLNGKEYKCKVSNKGLPSSIEKTISKAKGQPREPQVYTLPPSQEEMTKNQVSLTCLVKGFYPSDIAVEWESNGQPENNYKTTPPVLDSDGSFFLYSRLTVDKSRWQEGNVFSCSVMHEALHNHYTQKSLSLSLGK

SEQ ID NO: 29 - protein, 5 aa, Artificial Sequence
  VHCDRl
TYAMN

SEQ ID NO: 30 - protein, 19 aa, Artificial Sequence
  VHCDR2
RIRSKYNNYATYYADSVKD

SEQ ID NO: 31 - protein, 14 aa, Artificial Sequence
  VHCDR3
HGNFGNSYVSWFAY

SEQ ID NO: 32 - protein, 13 aa, Artificial Sequence
  VLCDR1
RSSTGAVTTSNYA

SEQ ID NO: 33 - protein, 7 aa, Artificial Sequence
  VLCDR2
GTNKRAP

SEQ ID NO: 34 - protein, 9 aa, Artificial Sequence
  VLCDR3
ALWYSNLWV

SEQ ID NO: 35 - protein, 19 aa, Artificial Sequence
  VHCDR2
RIRSKYNNYETYYADSVKD

SEQ ID NO: 36 - protein, 14 aa, Artificial Sequence
  VHCDR3
HSNFGNGYVSWFAY

SEQ ID NO: 37 - protein, 7 aa, Artificial Sequence
  VLCDR2
GTNLRAP

SEQ ID NO: 38 - protein, 7 aa, Artificial Sequence
  VLCDR2
GTWLRAP

SEQ ID NO: 39 - protein, 9 aa, Artificial Sequence
  VLCDR3
ALWRSGGWV

SEQ ID NO: 40 - protein, 9 aa, Artificial Sequence
  VLCDR3
ALWNKGGWV

SEQ ID NO: 41 - protein, 9 aa, Artificial Sequence
  VLCDR3
ALWNSGGWV

SEQ ID NO: 42 - protein, 205 aa, Artificial Sequence
  IL-15~IL-15Ra
NWVNVISDLKKIEDLIQSMHIDATLYTESDVHPSCKVTAMKCFLLELQVISCESGDASIHDTVENLIILANNSLSSNGNVTESGCKECEELEEKNIKEFLQSFVHIVQMFINTSSGGGSGGGGSGGGGSGGGGSGGGSGGITCPPPMSVEHADIWVKSYSLYSRERYICNSGFKRKAGTCSLTECVLNKATNVAHWTTPSLKCIR

SEQ ID NO: 43 - protein, 199 aa, Artificial Sequence
  IL-15~IL-15Ra
ITCPPPMSVEHADIWVKSYSLYSRERYICNSGFKRKAGTCSLTECVLNKATNVAHWTTPSLKCIRSGGSGGGGSGGGSGGGGSLQNWVNVISDLKKIEDLIQSMHIDATLYTESDVHPSCKVTAMKCFLLELQVISCESGDASIHDTVENLIILANNSLSSNGNVTESGCKECEELEEKNIKEFLQSFVHIVQMFINTS

SEQ ID NO: 44 - protein, 115 aa, Artificial Sequence
  IL-15
NWVNVISDLKKIEDLIQSMHIDATLYTESDVHPSCKVTAMKCFLLELQVISCESGDASIHDTVENLIILANNSLSSNGNVTESGCKECEELEEKNIKEFLQSFVHIVQMFINTSS

SEQ ID NO: 45 - protein, 65 aa, Artificial Sequence
  IL-15Ra
ITCPPPMSVEHADIWVKSYSLYSRERYICNSGFKRKAGTCSLTECVLNKATNVAHWTTPSLKCIR